European Patent Application EP 4 631 968 A1, published October 15, 2025. Title: Peptide for cartilage regeneration and uses thereof. Applicant: CAREGEN CO., LTD. The sequence listing filed with the application follows.

SEQUENCE LISTING (20 sequences)

SEQ ID NO: 1 - protein, 13 aa, synthetic construct
KVSYAAEKNRKNY

SEQ ID NO: 2 - protein, 5 aa, synthetic construct
SSFYF

SEQ ID NO: 3 - DNA, 23 bp, synthetic construct
  source 1..23: mol_type = other DNA
ctatctggacgaagcagctggca

SEQ ID NO: 4 - DNA, 22 bp, synthetic construct
  source 1..22: mol_type = other DNA
atgggtgcaatgtcaatgatgg

SEQ ID NO: 5 - DNA, 20 bp, synthetic construct
  source 1..20: mol_type = other DNA
aactcagggcaggaggatgt

SEQ ID NO: 6 - DNA, 20 bp, synthetic construct
  source 1..20: mol_type = other DNA
tgtccttttggtcgtcgttc

SEQ ID NO: 7 - DNA, 20 bp, synthetic construct
  source 1..20: mol_type = other DNA
ccagcccgaacttgtaaaga

SEQ ID NO: 8 - DNA, 20 bp, synthetic construct
  source 1..20: mol_type = other DNA
tggacgcacaaccatcatac

SEQ ID NO: 9 - DNA, 20 bp, synthetic construct
  source 1..20: mol_type = other DNA
gcaggctatgagcagtgtga

SEQ ID NO: 10 - DNA, 20 bp, synthetic construct
  source 1..20: mol_type = other DNA
gcatacctcggaagcagaag

SEQ ID NO: 11 - DNA, 20 bp, synthetic construct
  source 1..20: mol_type = other DNA
accacagtccatgccatcac

SEQ ID NO: 12 - DNA, 20 bp, synthetic construct
  source 1..20: mol_type = other DNA
tccaccaccctgttgctgta

SEQ ID NO: 13 - DNA, 20 bp, synthetic construct
  source 1..20: mol_type = other DNA
gcggaggaagtcggtgaaga

SEQ ID NO: 14 - DNA, 20 bp, synthetic construct
  source 1..20: mol_type = other DNA
ccctctcgcttcaggtcagc

SEQ ID NO: 15 - DNA, 23 bp, synthetic construct
  source 1..23: mol_type = other DNA
ctatctggacgaagcagctggca

SEQ ID NO: 16 - DNA, 22 bp, synthetic construct
  source 1..22: mol_type = other DNA
atgggtgcaatgtcaatgatgg

SEQ ID NO: 17 - DNA, 20 bp, synthetic construct
  source 1..20: mol_type = other DNA
aactcagggcaggaggatgt

SEQ ID NO: 18 - DNA, 20 bp, synthetic construct
  source 1..20: mol_type = other DNA
tgtccttttggtcgtcgttc

SEQ ID NO: 19 - DNA, 20 bp, synthetic construct
  source 1..20: mol_type = other DNA
tgagtcctcaagcctcctgt

SEQ ID NO: 20 - DNA, 20 bp, synthetic construct
  source 1..20: mol_type = other DNA
gtgccagatcatcaccacac